European Patent Application EP 4 461 130 A2, published November 13, 2024. Title: NOVEL INSECT RESISTANT GENES AND METHODS OF USE. Applicant: BASF SE. The sequence listing filed with the application follows.

SEQUENCE LISTING (36 sequences)

SEQ ID NO: 1 - DNA, 948 bp, synthetic construct
  misc_feature 1..948: note = Variant: Axmi486-R60S
  source 1..948: mol_type = other DNA
atgctggctgttgctgccaagacagagaacaacaaggagcagcaagtgatcacccacttcaaccagagggagaacaagttccctgatgttggccaaggaatccaatggctctctcagttctatgggaaatcattgaagaacaatggagaaggatattctcttggccaagatgtgatgagttacttcttggaggtgaagaacagctatgggcagcttgcaatggagcctcaggtcatctcaacaactcctctctgggctggccaaagtgatttggagaatgcaacagatcatgagcaaaccctcaactcaacagagttcaagaagacatacagcaacaccacaacaacctccacagagaatggcttcatgattggccaagaaacagaagggaaggttgggattccctttgttgctgaagggaaggtcaccatcaagacagagtacaacttcaatcacaccaatggctatgaaacttcagagagtgtggaatatattgctccaagccaaagcatcaaggttcctcctcacaccattgcaagggtgactgctctgctggatgtgaagaagatcaaggggaagatgcacctctattcagagattggcttgaacaaggattatggctatgacatggtgccactggtgtacaagtatggaggccccttcaagtatgtcacccttggaaccctctatgatgaaggctacaagcaagctcagctggattacttcaacatggggaatgtgattccagaagagattgaaactgtttcaaagagcaacaacccaaaccacttgctggcttctggtgttgggatctttgagagtgaatatggaagtgtcttcaatgtgaaggtggaatacatcaacattaacaccaagaagattgagaagacagagaatctcaccattgagccaaccattgtgccagtgaagcagaccaacaccaagtaa

SEQ ID NO: 2 - DNA, 948 bp, synthetic construct
  misc_feature 1..948: note = Variant: Axmi486-R60T
  source 1..948: mol_type = other DNA
atgctggctgttgctgccaagacagagaacaacaaggagcagcaagtgatcacccacttcaaccagagggagaacaagttccctgatgttggccaaggaatccaatggctctctcagttctatgggaaatcattgaagaacaatggagaaggatattctcttggccaagatgtgatgacgtacttcttggaggtgaagaacagctatgggcagcttgcaatggagcctcaggtcatctcaacaactcctctctgggctggccaaagtgatttggagaatgcaacagatcatgagcaaaccctcaactcaacagagttcaagaagacatacagcaacaccacaacaacctccacagagaatggcttcatgattggccaagaaacagaagggaaggttgggattccctttgttgctgaagggaaggtcaccatcaagacagagtacaacttcaatcacaccaatggctatgaaacttcagagagtgtggaatatattgctccaagccaaagcatcaaggttcctcctcacaccattgcaagggtgactgctctgctggatgtgaagaagatcaaggggaagatgcacctctattcagagattggcttgaacaaggattatggctatgacatggtgccactggtgtacaagtatggaggccccttcaagtatgtcacccttggaaccctctatgatgaaggctacaagcaagctcagctggattacttcaacatggggaatgtgattccagaagagattgaaactgtttcaaagagcaacaacccaaaccacttgctggcttctggtgttgggatctttgagagtgaatatggaagtgtcttcaatgtgaaggtggaatacatcaacattaacaccaagaagattgagaagacagagaatctcaccattgagccaaccattgtgccagtgaagcagaccaacaccaagtaa

SEQ ID NO: 3 - DNA, 948 bp, synthetic construct
  misc_feature 1..948: note = Variant: Axmi486-E275D
  source 1..948: mol_type = other DNA
atgctggctgttgctgccaagacagagaacaacaaggagcagcaagtgatcacccacttcaaccagagggagaacaagttccctgatgttggccaaggaatccaatggctctctcagttctatgggaaatcattgaagaacaatggagaaggatattctcttggccaagatgtgatgagatacttcttggaggtgaagaacagctatgggcagcttgcaatggagcctcaggtcatctcaacaactcctctctgggctggccaaagtgatttggagaatgcaacagatcatgagcaaaccctcaactcaacagagttcaagaagacatacagcaacaccacaacaacctccacagagaatggcttcatgattggccaagaaacagaagggaaggttgggattccctttgttgctgaagggaaggtcaccatcaagacagagtacaacttcaatcacaccaatggctatgaaacttcagagagtgtggaatatattgctccaagccaaagcatcaaggttcctcctcacaccattgcaagggtgactgctctgctggatgtgaagaagatcaaggggaagatgcacctctattcagagattggcttgaacaaggattatggctatgacatggtgccactggtgtacaagtatggaggccccttcaagtatgtcacccttggaaccctctatgatgaaggctacaagcaagctcagctggattacttcaacatggggaatgtgattccagaagagattgaaactgtttcaaagagcaacaacccaaaccacttgctggcttctggtgttgggatctttgagagtgattatggaagtgtcttcaatgtgaaggtggaatacatcaacattaacaccaagaagattgagaagacagagaatctcaccattgagccaaccattgtgccagtgaagcagaccaacaccaagtaa

SEQ ID NO: 4 - DNA, 948 bp, synthetic construct
  misc_feature 1..948: note = Variant: Axmi486-R60S E275D
  source 1..948: mol_type = other DNA
atgctggctgttgctgccaagacagagaacaacaaggagcagcaagtgatcacccacttcaaccagagggagaacaagttccctgatgttggccaaggaatccaatggctctctcagttctatgggaaatcattgaagaacaatggagaaggatattctcttggccaagatgtgatgagttacttcttggaggtgaagaacagctatgggcagcttgcaatggagcctcaggtcatctcaacaactcctctctgggctggccaaagtgatttggagaatgcaacagatcatgagcaaaccctcaactcaacagagttcaagaagacatacagcaacaccacaacaacctccacagagaatggcttcatgattggccaagaaacagaagggaaggttgggattccctttgttgctgaagggaaggtcaccatcaagacagagtacaacttcaatcacaccaatggctatgaaacttcagagagtgtggaatatattgctccaagccaaagcatcaaggttcctcctcacaccattgcaagggtgactgctctgctggatgtgaagaagatcaaggggaagatgcacctctattcagagattggcttgaacaaggattatggctatgacatggtgccactggtgtacaagtatggaggccccttcaagtatgtcacccttggaaccctctatgatgaaggctacaagcaagctcagctggattacttcaacatggggaatgtgattccagaagagattgaaactgtttcaaagagcaacaacccaaaccacttgctggcttctggtgttgggatctttgagagtgattatggaagtgtcttcaatgtgaaggtggaatacatcaacattaacaccaagaagattgagaagacagagaatctcaccattgagccaaccattgtgccagtgaagcagaccaacaccaagtaa

SEQ ID NO: 5 - DNA, 948 bp, synthetic construct
  misc_feature 1..948: note = Variant: Axmi486-R60T E275D
  source 1..948: mol_type = other DNA
atgctggctgttgctgccaagacagagaacaacaaggagcagcaagtgatcacccacttcaaccagagggagaacaagttccctgatgttggccaaggaatccaatggctctctcagttctatgggaaatcattgaagaacaatggagaaggatattctcttggccaagatgtgatgacgtacttcttggaggtgaagaacagctatgggcagcttgcaatggagcctcaggtcatctcaacaactcctctctgggctggccaaagtgatttggagaatgcaacagatcatgagcaaaccctcaactcaacagagttcaagaagacatacagcaacaccacaacaacctccacagagaatggcttcatgattggccaagaaacagaagggaaggttgggattccctttgttgctgaagggaaggtcaccatcaagacagagtacaacttcaatcacaccaatggctatgaaacttcagagagtgtggaatatattgctccaagccaaagcatcaaggttcctcctcacaccattgcaagggtgactgctctgctggatgtgaagaagatcaaggggaagatgcacctctattcagagattggcttgaacaaggattatggctatgacatggtgccactggtgtacaagtatggaggccccttcaagtatgtcacccttggaaccctctatgatgaaggctacaagcaagctcagctggattacttcaacatggggaatgtgattccagaagagattgaaactgtttcaaagagcaacaacccaaaccacttgctggcttctggtgttgggatctttgagagtgattatggaagtgtcttcaatgtgaaggtggaatacatcaacattaacaccaagaagattgagaagacagagaatctcaccattgagccaaccattgtgccagtgaagcagaccaacaccaagtaa

SEQ ID NO: 6 - DNA, 948 bp, synthetic construct
  misc_feature 1..948: note = Variant: Axmi486-R60S H97L T100N D96P
  source 1..948: mol_type = other DNA
atgctggctgttgctgccaagacagagaacaacaaggagcagcaagtgatcacccacttcaaccagagggagaacaagttccctgatgttggccaaggaatccaatggctctctcagttctatgggaaatcattgaagaacaatggagaaggatattctcttggccaagatgtgatgagttacttcttggaggtgaagaacagctatgggcagcttgcaatggagcctcaggtcatctcaacaactcctctctgggctggccaaagtgatttggagaatgcaacaccgctggagcaaaatctcaactcaacagagttcaagaagacatacagcaacaccacaacaacctccacagagaatggcttcatgattggccaagaaacagaagggaaggttgggattccctttgttgctgaagggaaggtcaccatcaagacagagtacaacttcaatcacaccaatggctatgaaacttcagagagtgtggaatatattgctccaagccaaagcatcaaggttcctcctcacaccattgcaagggtgactgctctgctggatgtgaagaagatcaaggggaagatgcacctctattcagagattggcttgaacaaggattatggctatgacatggtgccactggtgtacaagtatggaggccccttcaagtatgtcacccttggaaccctctatgatgaaggctacaagcaagctcagctggattacttcaacatggggaatgtgattccagaagagattgaaactgtttcaaagagcaacaacccaaaccacttgctggcttctggtgttgggatctttgagagtgaatatggaagtgtcttcaatgtgaaggtggaatacatcaacattaacaccaagaagattgagaagacagagaatctcaccattgagccaaccattgtgccagtgaagcagaccaacaccaagtaa

SEQ ID NO: 7 - DNA, 948 bp, synthetic construct
  misc_feature 1..948: note = Variant: Axmi486-R60T H97L T100N D96P
  source 1..948: mol_type = other DNA
atgctggctgttgctgccaagacagagaacaacaaggagcagcaagtgatcacccacttcaaccagagggagaacaagttccctgatgttggccaaggaatccaatggctctctcagttctatgggaaatcattgaagaacaatggagaaggatattctcttggccaagatgtgatgacgtacttcttggaggtgaagaacagctatgggcagcttgcaatggagcctcaggtcatctcaacaactcctctctgggctggccaaagtgatttggagaatgcaacaccgctggagcaaaatctcaactcaacagagttcaagaagacatacagcaacaccacaacaacctccacagagaatggcttcatgattggccaagaaacagaagggaaggttgggattccctttgttgctgaagggaaggtcaccatcaagacagagtacaacttcaatcacaccaatggctatgaaacttcagagagtgtggaatatattgctccaagccaaagcatcaaggttcctcctcacaccattgcaagggtgactgctctgctggatgtgaagaagatcaaggggaagatgcacctctattcagagattggcttgaacaaggattatggctatgacatggtgccactggtgtacaagtatggaggccccttcaagtatgtcacccttggaaccctctatgatgaaggctacaagcaagctcagctggattacttcaacatggggaatgtgattccagaagagattgaaactgtttcaaagagcaacaacccaaaccacttgctggcttctggtgttgggatctttgagagtgaatatggaagtgtcttcaatgtgaaggtggaatacatcaacattaacaccaagaagattgagaagacagagaatctcaccattgagccaaccattgtgccagtgaagcagaccaacaccaagtaa

SEQ ID NO: 8 - DNA, 948 bp, synthetic construct
  misc_feature 1..948: note = Variant: Axmi486-E275D H97L T100N D96P
  source 1..948: mol_type = other DNA
atgctggctgttgctgccaagacagagaacaacaaggagcagcaagtgatcacccacttcaaccagagggagaacaagttccctgatgttggccaaggaatccaatggctctctcagttctatgggaaatcattgaagaacaatggagaaggatattctcttggccaagatgtgatgagatacttcttggaggtgaagaacagctatgggcagcttgcaatggagcctcaggtcatctcaacaactcctctctgggctggccaaagtgatttggagaatgcaacaccgctggagcaaaatctcaactcaacagagttcaagaagacatacagcaacaccacaacaacctccacagagaatggcttcatgattggccaagaaacagaagggaaggttgggattccctttgttgctgaagggaaggtcaccatcaagacagagtacaacttcaatcacaccaatggctatgaaacttcagagagtgtggaatatattgctccaagccaaagcatcaaggttcctcctcacaccattgcaagggtgactgctctgctggatgtgaagaagatcaaggggaagatgcacctctattcagagattggcttgaacaaggattatggctatgacatggtgccactggtgtacaagtatggaggccccttcaagtatgtcacccttggaaccctctatgatgaaggctacaagcaagctcagctggattacttcaacatggggaatgtgattccagaagagattgaaactgtttcaaagagcaacaacccaaaccacttgctggcttctggtgttgggatctttgagagtgattatggaagtgtcttcaatgtgaaggtggaatacatcaacattaacaccaagaagattgagaagacagagaatctcaccattgagccaaccattgtgccagtgaagcagaccaacaccaagtaa

SEQ ID NO: 9 - DNA, 948 bp, synthetic construct
  misc_feature 1..948: note = Variant: Axmi486-R60S E275D H97L T100N D96P
  source 1..948: mol_type = other DNA
atgctggctgttgctgccaagacagagaacaacaaggagcagcaagtgatcacccacttcaaccagagggagaacaagttccctgatgttggccaaggaatccaatggctctctcagttctatgggaaatcattgaagaacaatggagaaggatattctcttggccaagatgtgatgagttacttcttggaggtgaagaacagctatgggcagcttgcaatggagcctcaggtcatctcaacaactcctctctgggctggccaaagtgatttggagaatgcaacaccgctggagcaaaatctcaactcaacagagttcaagaagacatacagcaacaccacaacaacctccacagagaatggcttcatgattggccaagaaacagaagggaaggttgggattccctttgttgctgaagggaaggtcaccatcaagacagagtacaacttcaatcacaccaatggctatgaaacttcagagagtgtggaatatattgctccaagccaaagcatcaaggttcctcctcacaccattgcaagggtgactgctctgctggatgtgaagaagatcaaggggaagatgcacctctattcagagattggcttgaacaaggattatggctatgacatggtgccactggtgtacaagtatggaggccccttcaagtatgtcacccttggaaccctctatgatgaaggctacaagcaagctcagctggattacttcaacatggggaatgtgattccagaagagattgaaactgtttcaaagagcaacaacccaaaccacttgctggcttctggtgttgggatctttgagagtgattatggaagtgtcttcaatgtgaaggtggaatacatcaacattaacaccaagaagattgagaagacagagaatctcaccattgagccaaccattgtgccagtgaagcagaccaacaccaagtaa

SEQ ID NO: 10 - DNA, 948 bp, synthetic construct
  misc_feature 1..948: note = Variant: Axmi486-R60T E275D H97L T100N D96P
  source 1..948: mol_type = other DNA
atgctggctgttgctgccaagacagagaacaacaaggagcagcaagtgatcacccacttcaaccagagggagaacaagttccctgatgttggccaaggaatccaatggctctctcagttctatgggaaatcattgaagaacaatggagaaggatattctcttggccaagatgtgatgacgtacttcttggaggtgaagaacagctatgggcagcttgcaatggagcctcaggtcatctcaacaactcctctctgggctggccaaagtgatttggagaatgcaacaccgctggagcaaaatctcaactcaacagagttcaagaagacatacagcaacaccacaacaacctccacagagaatggcttcatgattggccaagaaacagaagggaaggttgggattccctttgttgctgaagggaaggtcaccatcaagacagagtacaacttcaatcacaccaatggctatgaaacttcagagagtgtggaatatattgctccaagccaaagcatcaaggttcctcctcacaccattgcaagggtgactgctctgctggatgtgaagaagatcaaggggaagatgcacctctattcagagattggcttgaacaaggattatggctatgacatggtgccactggtgtacaagtatggaggccccttcaagtatgtcacccttggaaccctctatgatgaaggctacaagcaagctcagctggattacttcaacatggggaatgtgattccagaagagattgaaactgtttcaaagagcaacaacccaaaccacttgctggcttctggtgttgggatctttgagagtgattatggaagtgtcttcaatgtgaaggtggaatacatcaacattaacaccaagaagattgagaagacagagaatctcaccattgagccaaccattgtgccagtgaagcagaccaacaccaagtaa

SEQ ID NO: 11 - DNA, 948 bp, synthetic construct
  misc_feature 1..948: note = Variant: Axmi486-R60S T100N D96P
  source 1..948: mol_type = other DNA
atgctggctgttgctgccaagacagagaacaacaaggagcagcaagtgatcacccacttcaaccagagggagaacaagttccctgatgttggccaaggaatccaatggctctctcagttctatgggaaatcattgaagaacaatggagaaggatattctcttggccaagatgtgatgagttacttcttggaggtgaagaacagctatgggcagcttgcaatggagcctcaggtcatctcaacaactcctctctgggctggccaaagtgatttggagaatgcaacaccgcatgagcaaaatctcaactcaacagagttcaagaagacatacagcaacaccacaacaacctccacagagaatggcttcatgattggccaagaaacagaagggaaggttgggattccctttgttgctgaagggaaggtcaccatcaagacagagtacaacttcaatcacaccaatggctatgaaacttcagagagtgtggaatatattgctccaagccaaagcatcaaggttcctcctcacaccattgcaagggtgactgctctgctggatgtgaagaagatcaaggggaagatgcacctctattcagagattggcttgaacaaggattatggctatgacatggtgccactggtgtacaagtatggaggccccttcaagtatgtcacccttggaaccctctatgatgaaggctacaagcaagctcagctggattacttcaacatggggaatgtgattccagaagagattgaaactgtttcaaagagcaacaacccaaaccacttgctggcttctggtgttgggatctttgagagtgaatatggaagtgtcttcaatgtgaaggtggaatacatcaacattaacaccaagaagattgagaagacagagaatctcaccattgagccaaccattgtgccagtgaagcagaccaacaccaagtaa

SEQ ID NO: 12 - DNA, 948 bp, synthetic construct
  misc_feature 1..948: note = Variant: Axmi486-R60T T100N D96P
  source 1..948: mol_type = other DNA
atgctggctgttgctgccaagacagagaacaacaaggagcagcaagtgatcacccacttcaaccagagggagaacaagttccctgatgttggccaaggaatccaatggctctctcagttctatgggaaatcattgaagaacaatggagaaggatattctcttggccaagatgtgatgacgtacttcttggaggtgaagaacagctatgggcagcttgcaatggagcctcaggtcatctcaacaactcctctctgggctggccaaagtgatttggagaatgcaacaccgcatgagcaaaatctcaactcaacagagttcaagaagacatacagcaacaccacaacaacctccacagagaatggcttcatgattggccaagaaacagaagggaaggttgggattccctttgttgctgaagggaaggtcaccatcaagacagagtacaacttcaatcacaccaatggctatgaaacttcagagagtgtggaatatattgctccaagccaaagcatcaaggttcctcctcacaccattgcaagggtgactgctctgctggatgtgaagaagatcaaggggaagatgcacctctattcagagattggcttgaacaaggattatggctatgacatggtgccactggtgtacaagtatggaggccccttcaagtatgtcacccttggaaccctctatgatgaaggctacaagcaagctcagctggattacttcaacatggggaatgtgattccagaagagattgaaactgtttcaaagagcaacaacccaaaccacttgctggcttctggtgttgggatctttgagagtgaatatggaagtgtcttcaatgtgaaggtggaatacatcaacattaacaccaagaagattgagaagacagagaatctcaccattgagccaaccattgtgccagtgaagcagaccaacaccaagtaa

SEQ ID NO: 13 - DNA, 948 bp, synthetic construct
  misc_feature 1..948: note = Variant: Axmi486-E275D T100N D96P
  source 1..948: mol_type = other DNA
atgctggctgttgctgccaagacagagaacaacaaggagcagcaagtgatcacccacttcaaccagagggagaacaagttccctgatgttggccaaggaatccaatggctctctcagttctatgggaaatcattgaagaacaatggagaaggatattctcttggccaagatgtgatgagatacttcttggaggtgaagaacagctatgggcagcttgcaatggagcctcaggtcatctcaacaactcctctctgggctggccaaagtgatttggagaatgcaacaccgcatgagcaaaatctcaactcaacagagttcaagaagacatacagcaacaccacaacaacctccacagagaatggcttcatgattggccaagaaacagaagggaaggttgggattccctttgttgctgaagggaaggtcaccatcaagacagagtacaacttcaatcacaccaatggctatgaaacttcagagagtgtggaatatattgctccaagccaaagcatcaaggttcctcctcacaccattgcaagggtgactgctctgctggatgtgaagaagatcaaggggaagatgcacctctattcagagattggcttgaacaaggattatggctatgacatggtgccactggtgtacaagtatggaggccccttcaagtatgtcacccttggaaccctctatgatgaaggctacaagcaagctcagctggattacttcaacatggggaatgtgattccagaagagattgaaactgtttcaaagagcaacaacccaaaccacttgctggcttctggtgttgggatctttgagagtgattatggaagtgtcttcaatgtgaaggtggaatacatcaacattaacaccaagaagattgagaagacagagaatctcaccattgagccaaccattgtgccagtgaagcagaccaacaccaagtaa

SEQ ID NO: 14 - DNA, 948 bp, synthetic construct
  misc_feature 1..948: note = Variant: Axmi486-R60S E275D T100N D96P
  source 1..948: mol_type = other DNA
atgctggctgttgctgccaagacagagaacaacaaggagcagcaagtgatcacccacttcaaccagagggagaacaagttccctgatgttggccaaggaatccaatggctctctcagttctatgggaaatcattgaagaacaatggagaaggatattctcttggccaagatgtgatgagttacttcttggaggtgaagaacagctatgggcagcttgcaatggagcctcaggtcatctcaacaactcctctctgggctggccaaagtgatttggagaatgcaacaccgcatgagcaaaatctcaactcaacagagttcaagaagacatacagcaacaccacaacaacctccacagagaatggcttcatgattggccaagaaacagaagggaaggttgggattccctttgttgctgaagggaaggtcaccatcaagacagagtacaacttcaatcacaccaatggctatgaaacttcagagagtgtggaatatattgctccaagccaaagcatcaaggttcctcctcacaccattgcaagggtgactgctctgctggatgtgaagaagatcaaggggaagatgcacctctattcagagattggcttgaacaaggattatggctatgacatggtgccactggtgtacaagtatggaggccccttcaagtatgtcacccttggaaccctctatgatgaaggctacaagcaagctcagctggattacttcaacatggggaatgtgattccagaagagattgaaactgtttcaaagagcaacaacccaaaccacttgctggcttctggtgttgggatctttgagagtgattatggaagtgtcttcaatgtgaaggtggaatacatcaacattaacaccaagaagattgagaagacagagaatctcaccattgagccaaccattgtgccagtgaagcagaccaacaccaagtaa

SEQ ID NO: 15 - DNA, 948 bp, synthetic construct
  misc_feature 1..948: note = Variant: Axmi486-R60T E275D T100N D96P
  source 1..948: mol_type = other DNA
atgctggctgttgctgccaagacagagaacaacaaggagcagcaagtgatcacccacttcaaccagagggagaacaagttccctgatgttggccaaggaatccaatggctctctcagttctatgggaaatcattgaagaacaatggagaaggatattctcttggccaagatgtgatgacgtacttcttggaggtgaagaacagctatgggcagcttgcaatggagcctcaggtcatctcaacaactcctctctgggctggccaaagtgatttggagaatgcaacaccgcatgagcaaaatctcaactcaacagagttcaagaagacatacagcaacaccacaacaacctccacagagaatggcttcatgattggccaagaaacagaagggaaggttgggattccctttgttgctgaagggaaggtcaccatcaagacagagtacaacttcaatcacaccaatggctatgaaacttcagagagtgtggaatatattgctccaagccaaagcatcaaggttcctcctcacaccattgcaagggtgactgctctgctggatgtgaagaagatcaaggggaagatgcacctctattcagagattggcttgaacaaggattatggctatgacatggtgccactggtgtacaagtatggaggccccttcaagtatgtcacccttggaaccctctatgatgaaggctacaagcaagctcagctggattacttcaacatggggaatgtgattccagaagagattgaaactgtttcaaagagcaacaacccaaaccacttgctggcttctggtgttgggatctttgagagtgattatggaagtgtcttcaatgtgaaggtggaatacatcaacattaacaccaagaagattgagaagacagagaatctcaccattgagccaaccattgtgccagtgaagcagaccaacaccaagtaa

SEQ ID NO: 16 - protein, 315 aa, synthetic construct
  REGION 1..315: note = Variant: Axmi486-R60S
MLAVAAKTENNKEQQVITHFNQRENKFPDVGQGIQWLSQFYGKSLKNNGEGYSLGQDVMSYFLEVKNSYGQLAMEPQVISTTPLWAGQSDLENATDHEQTLNSTEFKKTYSNTTTTSTENGFMIGQETEGKVGIPFVAEGKVTIKTEYNFNHTNGYETSESVEYIAPSQSIKVPPHTIARVTALLDVKKIKGKMHLYSEIGLNKDYGYDMVPLVYKYGGPFKYVTLGTLYDEGYKQAQLDYFNMGNVIPEEIETVSKSNNPNHLLASGVGIFESEYGSVFNVKVEYININTKKIEKTENLTIEPTIVPVKQTNTK

SEQ ID NO: 17 - protein, 315 aa, synthetic construct
  REGION 1..315: note = Variant: Axmi486-R60T
MLAVAAKTENNKEQQVITHFNQRENKFPDVGQGIQWLSQFYGKSLKNNGEGYSLGQDVMTYFLEVKNSYGQLAMEPQVISTTPLWAGQSDLENATDHEQTLNSTEFKKTYSNTTTTSTENGFMIGQETEGKVGIPFVAEGKVTIKTEYNFNHTNGYETSESVEYIAPSQSIKVPPHTIARVTALLDVKKIKGKMHLYSEIGLNKDYGYDMVPLVYKYGGPFKYVTLGTLYDEGYKQAQLDYFNMGNVIPEEIETVSKSNNPNHLLASGVGIFESEYGSVFNVKVEYININTKKIEKTENLTIEPTIVPVKQTNTK

SEQ ID NO: 18 - protein, 315 aa, synthetic construct
  REGION 1..315: note = Variant: Axmi486-E275D
MLAVAAKTENNKEQQVITHFNQRENKFPDVGQGIQWLSQFYGKSLKNNGEGYSLGQDVMRYFLEVKNSYGQLAMEPQVISTTPLWAGQSDLENATDHEQTLNSTEFKKTYSNTTTTSTENGFMIGQETEGKVGIPFVAEGKVTIKTEYNFNHTNGYETSESVEYIAPSQSIKVPPHTIARVTALLDVKKIKGKMHLYSEIGLNKDYGYDMVPLVYKYGGPFKYVTLGTLYDEGYKQAQLDYFNMGNVIPEEIETVSKSNNPNHLLASGVGIFESDYGSVFNVKVEYININTKKIEKTENLTIEPTIVPVKQTNTK

SEQ ID NO: 19 - protein, 315 aa, synthetic construct
  REGION 1..315: note = Variant: Axmi486-R60S E275D
MLAVAAKTENNKEQQVITHFNQRENKFPDVGQGIQWLSQFYGKSLKNNGEGYSLGQDVMSYFLEVKNSYGQLAMEPQVISTTPLWAGQSDLENATDHEQTLNSTEFKKTYSNTTTTSTENGFMIGQETEGKVGIPFVAEGKVTIKTEYNFNHTNGYETSESVEYIAPSQSIKVPPHTIARVTALLDVKKIKGKMHLYSEIGLNKDYGYDMVPLVYKYGGPFKYVTLGTLYDEGYKQAQLDYFNMGNVIPEEIETVSKSNNPNHLLASGVGIFESDYGSVFNVKVEYININTKKIEKTENLTIEPTIVPVKQTNTK

SEQ ID NO: 20 - protein, 315 aa, synthetic construct
  REGION 1..315: note = Variant: Axmi486-R60T E275D
MLAVAAKTENNKEQQVITHFNQRENKFPDVGQGIQWLSQFYGKSLKNNGEGYSLGQDVMTYFLEVKNSYGQLAMEPQVISTTPLWAGQSDLENATDHEQTLNSTEFKKTYSNTTTTSTENGFMIGQETEGKVGIPFVAEGKVTIKTEYNFNHTNGYETSESVEYIAPSQSIKVPPHTIARVTALLDVKKIKGKMHLYSEIGLNKDYGYDMVPLVYKYGGPFKYVTLGTLYDEGYKQAQLDYFNMGNVIPEEIETVSKSNNPNHLLASGVGIFESDYGSVFNVKVEYININTKKIEKTENLTIEPTIVPVKQTNTK

SEQ ID NO: 21 - protein, 315 aa, synthetic construct
  REGION 1..315: note = Variant: Axmi486-R60S H97L T100N D96P
MLAVAAKTENNKEQQVITHFNQRENKFPDVGQGIQWLSQFYGKSLKNNGEGYSLGQDVMSYFLEVKNSYGQLAMEPQVISTTPLWAGQSDLENATPLEQNLNSTEFKKTYSNTTTTSTENGFMIGQETEGKVGIPFVAEGKVTIKTEYNFNHTNGYETSESVEYIAPSQSIKVPPHTIARVTALLDVKKIKGKMHLYSEIGLNKDYGYDMVPLVYKYGGPFKYVTLGTLYDEGYKQAQLDYFNMGNVIPEEIETVSKSNNPNHLLASGVGIFESEYGSVFNVKVEYININTKKIEKTENLTIEPTIVPVKQTNTK

SEQ ID NO: 22 - protein, 315 aa, synthetic construct
  REGION 1..315: note = Variant: Axmi486-R60T H97L T100N D96P
MLAVAAKTENNKEQQVITHFNQRENKFPDVGQGIQWLSQFYGKSLKNNGEGYSLGQDVMTYFLEVKNSYGQLAMEPQVISTTPLWAGQSDLENATPLEQNLNSTEFKKTYSNTTTTSTENGFMIGQETEGKVGIPFVAEGKVTIKTEYNFNHTNGYETSESVEYIAPSQSIKVPPHTIARVTALLDVKKIKGKMHLYSEIGLNKDYGYDMVPLVYKYGGPFKYVTLGTLYDEGYKQAQLDYFNMGNVIPEEIETVSKSNNPNHLLASGVGIFESEYGSVFNVKVEYININTKKIEKTENLTIEPTIVPVKQTNTK

SEQ ID NO: 23 - protein, 315 aa, synthetic construct
  REGION 1..315: note = Variant: Axmi486-E275D H97L T100N D96P
MLAVAAKTENNKEQQVITHFNQRENKFPDVGQGIQWLSQFYGKSLKNNGEGYSLGQDVMRYFLEVKNSYGQLAMEPQVISTTPLWAGQSDLENATPLEQNLNSTEFKKTYSNTTTTSTENGFMIGQETEGKVGIPFVAEGKVTIKTEYNFNHTNGYETSESVEYIAPSQSIKVPPHTIARVTALLDVKKIKGKMHLYSEIGLNKDYGYDMVPLVYKYGGPFKYVTLGTLYDEGYKQAQLDYFNMGNVIPEEIETVSKSNNPNHLLASGVGIFESDYGSVFNVKVEYININTKKIEKTENLTIEPTIVPVKQTNTK

SEQ ID NO: 24 - protein, 315 aa, synthetic construct
  REGION 1..315: note = Variant: Axmi486-R60S E275D H97L T100N D96P
MLAVAAKTENNKEQQVITHFNQRENKFPDVGQGIQWLSQFYGKSLKNNGEGYSLGQDVMSYFLEVKNSYGQLAMEPQVISTTPLWAGQSDLENATPLEQNLNSTEFKKTYSNTTTTSTENGFMIGQETEGKVGIPFVAEGKVTIKTEYNFNHTNGYETSESVEYIAPSQSIKVPPHTIARVTALLDVKKIKGKMHLYSEIGLNKDYGYDMVPLVYKYGGPFKYVTLGTLYDEGYKQAQLDYFNMGNVIPEEIETVSKSNNPNHLLASGVGIFESDYGSVFNVKVEYININTKKIEKTENLTIEPTIVPVKQTNTK

SEQ ID NO: 25 - protein, 315 aa, synthetic construct
  REGION 1..315: note = Variant: Axmi486-R60T E275D H97L T100N D96P
MLAVAAKTENNKEQQVITHFNQRENKFPDVGQGIQWLSQFYGKSLKNNGEGYSLGQDVMTYFLEVKNSYGQLAMEPQVISTTPLWAGQSDLENATPLEQNLNSTEFKKTYSNTTTTSTENGFMIGQETEGKVGIPFVAEGKVTIKTEYNFNHTNGYETSESVEYIAPSQSIKVPPHTIARVTALLDVKKIKGKMHLYSEIGLNKDYGYDMVPLVYKYGGPFKYVTLGTLYDEGYKQAQLDYFNMGNVIPEEIETVSKSNNPNHLLASGVGIFESDYGSVFNVKVEYININTKKIEKTENLTIEPTIVPVKQTNTK

SEQ ID NO: 26 - protein, 315 aa, synthetic construct
  REGION 1..315: note = Variant: Axmi486-R60S T100N D96P
MLAVAAKTENNKEQQVITHFNQRENKFPDVGQGIQWLSQFYGKSLKNNGEGYSLGQDVMSYFLEVKNSYGQLAMEPQVISTTPLWAGQSDLENATPHEQNLNSTEFKKTYSNTTTTSTENGFMIGQETEGKVGIPFVAEGKVTIKTEYNFNHTNGYETSESVEYIAPSQSIKVPPHTIARVTALLDVKKIKGKMHLYSEIGLNKDYGYDMVPLVYKYGGPFKYVTLGTLYDEGYKQAQLDYFNMGNVIPEEIETVSKSNNPNHLLASGVGIFESEYGSVFNVKVEYININTKKIEKTENLTIEPTIVPVKQTNTK

SEQ ID NO: 27 - protein, 315 aa, synthetic construct
  REGION 1..315: note = Variant: Axmi486-R60T T100N D96P
MLAVAAKTENNKEQQVITHFNQRENKFPDVGQGIQWLSQFYGKSLKNNGEGYSLGQDVMTYFLEVKNSYGQLAMEPQVISTTPLWAGQSDLENATPHEQNLNSTEFKKTYSNTTTTSTENGFMIGQETEGKVGIPFVAEGKVTIKTEYNFNHTNGYETSESVEYIAPSQSIKVPPHTIARVTALLDVKKIKGKMHLYSEIGLNKDYGYDMVPLVYKYGGPFKYVTLGTLYDEGYKQAQLDYFNMGNVIPEEIETVSKSNNPNHLLASGVGIFESEYGSVFNVKVEYININTKKIEKTENLTIEPTIVPVKQTNTK

SEQ ID NO: 28 - protein, 315 aa, synthetic construct
  REGION 1..315: note = Variant: Axmi486-E275D T100N D96P
MLAVAAKTENNKEQQVITHFNQRENKFPDVGQGIQWLSQFYGKSLKNNGEGYSLGQDVMRYFLEVKNSYGQLAMEPQVISTTPLWAGQSDLENATPHEQNLNSTEFKKTYSNTTTTSTENGFMIGQETEGKVGIPFVAEGKVTIKTEYNFNHTNGYETSESVEYIAPSQSIKVPPHTIARVTALLDVKKIKGKMHLYSEIGLNKDYGYDMVPLVYKYGGPFKYVTLGTLYDEGYKQAQLDYFNMGNVIPEEIETVSKSNNPNHLLASGVGIFESDYGSVFNVKVEYININTKKIEKTENLTIEPTIVPVKQTNTK

SEQ ID NO: 29 - protein, 315 aa, synthetic construct
  REGION 1..315: note = Variant: Axmi486-R60S E275D T100N D96P
MLAVAAKTENNKEQQVITHFNQRENKFPDVGQGIQWLSQFYGKSLKNNGEGYSLGQDVMSYFLEVKNSYGQLAMEPQVISTTPLWAGQSDLENATPHEQNLNSTEFKKTYSNTTTTSTENGFMIGQETEGKVGIPFVAEGKVTIKTEYNFNHTNGYETSESVEYIAPSQSIKVPPHTIARVTALLDVKKIKGKMHLYSEIGLNKDYGYDMVPLVYKYGGPFKYVTLGTLYDEGYKQAQLDYFNMGNVIPEEIETVSKSNNPNHLLASGVGIFESDYGSVFNVKVEYININTKKIEKTENLTIEPTIVPVKQTNTK

SEQ ID NO: 30 - protein, 315 aa, synthetic construct
  REGION 1..315: note = Variant: Axmi486-R60T E275D T100N D96P
MLAVAAKTENNKEQQVITHFNQRENKFPDVGQGIQWLSQFYGKSLKNNGEGYSLGQDVMTYFLEVKNSYGQLAMEPQVISTTPLWAGQSDLENATPHEQNLNSTEFKKTYSNTTTTSTENGFMIGQETEGKVGIPFVAEGKVTIKTEYNFNHTNGYETSESVEYIAPSQSIKVPPHTIARVTALLDVKKIKGKMHLYSEIGLNKDYGYDMVPLVYKYGGPFKYVTLGTLYDEGYKQAQLDYFNMGNVIPEEIETVSKSNNPNHLLASGVGIFESDYGSVFNVKVEYININTKKIEKTENLTIEPTIVPVKQTNTK

SEQ ID NO: 31 - DNA, 1023 bp, Bacillus thuringiensis
  misc_feature 1..1023: note = axmi-486 (Ref: WO/2015/088937)
  source 1..1023: mol_type = unassigned DNA
gtgagggagaaggatttgaataaaaaagtaacaaaggcagtattaagcatgatagtgggtataagtgttttagcatctcctttagctgtagccgcaaaaacagagaataataaagaacaacaagtaattacacattttaatcagagagaaaataagttccctgatgtaggacaggggattcaatggttatctcaattttatggaaagtctttaaagaataatggtgaaggatactccttaggtcaggatgtaatgagatattttttagaagtaaagaattcttacggtcaattggcaatggaacctcaagtaataagcactacacctctttgggccggccaaagtgacttggaaaatgcaactgatcatgaacaaactttaaattccacagaatttaaaaaaacgtattctaacacaacaaccacctctacagaaaatggatttatgataggtcaagagactgaagggaaagttggtattccctttgtcgcagaaggaaaagtcaccataaaaactgaatataactttaatcatactaatgggtatgaaacatctgaaagtgtagagtatattgctccttctcaatctattaaggtaccaccgcatactattgcccgagtgacagcattattagatgtgaaaaaaatcaaagggaaaatgcatctatattcagaaattgggcttaataaagattatggttacgatatggtgccacttgtttataaatatggaggtccatttaagtatgtaaccttaggcacattatatgacgagggctataagcaggcacaattagattatttcaatatgggaaatgttataccggaagaaattgagactgtttcaaaaagtaacaatcccaaccatttattagcaagtggagtaggaatctttgaatcagaatacggaagtgtatttaatgttaaagttgaatacattaatattaatacgaaaaagattgaaaaaacagagaatcttactattgaacctacaatagtccctgttaaacagacgaatacaaaa

SEQ ID NO: 32 - protein, 341 aa, Bacillus thuringiensis
  REGION 1..341: note = axmi-486 (Ref: WO/2015/088937)
MREKDLNKKVTKAVLSMIVGISVLASPLAVAAKTENNKEQQVITHFNQRENKFPDVGQGIQWLSQFYGKSLKNNGEGYSLGQDVMRYFLEVKNSYGQLAMEPQVISTTPLWAGQSDLENATDHEQTLNSTEFKKTYSNTTTTSTENGFMIGQETEGKVGIPFVAEGKVTIKTEYNFNHTNGYETSESVEYIAPSQSIKVPPHTIARVTALLDVKKIKGKMHLYSEIGLNKDYGYDMVPLVYKYGGPFKYVTLGTLYDEGYKQAQLDYFNMGNVIPEEIETVSKSNNPNHLLASGVGIFESEYGSVFNVKVEYININTKKIEKTENLTIEPTIVPVKQTNTK

SEQ ID NO: 33 - protein, 325 aa, Bacillus thuringiensis
  REGION 1..325: note = axmi-486 (alternate start site) (Ref: WO/2015/088937)
MIVGISVLASPLAVAAKTENNKEQQVITHFNQRENKFPDVGQGIQWLSQFYGKSLKNNGEGYSLGQDVMRYFLEVKNSYGQLAMEPQVISTTPLWAGQSDLENATDHEQTLNSTEFKKTYSNTTTTSTENGFMIGQETEGKVGIPFVAEGKVTIKTEYNFNHTNGYETSESVEYIAPSQSIKVPPHTIARVTALLDVKKIKGKMHLYSEIGLNKDYGYDMVPLVYKYGGPFKYVTLGTLYDEGYKQAQLDYFNMGNVIPEEIETVSKSNNPNHLLASGVGIFESEYGSVFNVKVEYININTKKIEKTENLTIEPTIVPVKQTNTK

SEQ ID NO: 34 - protein, 315 aa, Bacillus thuringiensis
  REGION 1..315: note = axmi-486 (alternate start site) (Ref: WO/2015/088937)
MLAVAAKTENNKEQQVITHFNQRENKFPDVGQGIQWLSQFYGKSLKNNGEGYSLGQDVMRYFLEVKNSYGQLAMEPQVISTTPLWAGQSDLENATDHEQTLNSTEFKKTYSNTTTTSTENGFMIGQETEGKVGIPFVAEGKVTIKTEYNFNHTNGYETSESVEYIAPSQSIKVPPHTIARVTALLDVKKIKGKMHLYSEIGLNKDYGYDMVPLVYKYGGPFKYVTLGTLYDEGYKQAQLDYFNMGNVIPEEIETVSKSNNPNHLLASGVGIFESEYGSVFNVKVEYININTKKIEKTENLTIEPTIVPVKQTNTK

SEQ ID NO: 35 - protein, 257 aa, Bacillus thuringiensis
  REGION 1..257: note = axmi-486 (alternate start site) (Ref: WO/2015/088937)
MRYFLEVKNSYGQLAMEPQVISTTPLWAGQSDLENATDHEQTLNSTEFKKTYSNTTTTSTENGFMIGQETEGKVGIPFVAEGKVTIKTEYNFNHTNGYETSESVEYIAPSQSIKVPPHTIARVTALLDVKKIKGKMHLYSEIGLNKDYGYDMVPLVYKYGGPFKYVTLGTLYDEGYKQAQLDYFNMGNVIPEEIETVSKSNNPNHLLASGVGIFESEYGSVFNVKVEYININTKKIEKTENLTIEPTIVPVKQTNTK

SEQ ID NO: 36 - protein, 242 aa, Bacillus thuringiensis
  REGION 1..242: note = axmi-486 (alternate start site) (Ref: WO/2015/088937)
MEPQVISTTPLWAGQSDLENATDHEQTLNSTEFKKTYSNTTTTSTENGFMIGQETEGKVGIPFVAEGKVTIKTEYNFNHTNGYETSESVEYIAPSQSIKVPPHTIARVTALLDVKKIKGKMHLYSEIGLNKDYGYDMVPLVYKYGGPFKYVTLGTLYDEGYKQAQLDYFNMGNVIPEEIETVSKSNNPNHLLASGVGIFESEYGSVFNVKVEYININTKKIEKTENLTIEPTIVPVKQTNTK